European Patent Specification EP 3 834 839 B1, published November 22, 2023. Title: Novel Artificial Tears Containing Recombinant Human Lysozyme. Applicant: SHAANXI HK BIOTECH CO. LTD. The sequence listing filed with the application follows.

SEQUENCE LISTING (4 sequences)

SEQ ID NO: 1 - protein, 130 aa, Human lysozyme
KVFERCELARTLKRLGMDGYRGISLANWMCLAKWESGYNTRATNYNAGDRSTDYGIFQINSRYWCNDGKTPGAVNACHLSCSALLQDNIADAVACAKRVVRDPQGIRAWVAWRNRCQNRDVRQYVQGCGV

SEQ ID NO: 2 - DNA, 411 bp, Artificial Sequence
ctcgagaaaagaaaggtctttgaaaggtgtgagttggccagaactctgaaaagattgggaatggatggctacaggggaatcagcctagcaaactggatgtgtttggccaaatgggagagtggttacaacacacgagctacaaactacaatgctggagacagaagcactgattatgggatatttcagatcaatagccgctactggtgtaatgatggcaaaaccccaggagcagttaatgcctgtcatttatcctgcagtgctttgctgcaagataacatcgctgatgctgtagcttgtgcaaagagggttgtccgtgatccacaaggcattagagcatgggtggcatggagaaatcgttgtcaaaacagagatgtccgtcagtatgttcaaggttgtggagtgtaagaattc

SEQ ID NO: 3 - DNA, 34 bp, Artificial Sequence
gcctcgagaaaagaaaggtctttgaaaggtgtga

SEQ ID NO: 4 - DNA, 28 bp, Artificial Sequence
cggaattcttacactccacaaccttgaa